European Patent Specification EP 3 525 583 B1, published July 23, 2025. Title: ANTI-C1s ANTIBODIES AND METHODS OF USE THEREOF. Applicant: BIOVERATIV USA INC. PANICKER, SANDIP PARRU, GRAHAM STAGLIANO, NANCY E. The sequence listing filed with the application follows.

SEQUENCE LISTING (54 sequences)

SEQ ID NO: 1 - protein, 15 aa, Artificial Sequence
  VL CDR1
KASQSVDYDGDSYMN

SEQ ID NO: 2 - protein, 7 aa, Artificial Sequence
  VL CDR2
DASNLES

SEQ ID NO: 3 - protein, 9 aa, Artificial Sequence
  VL CDR3
QQSNEDPWT

SEQ ID NO: 4 - protein, 5 aa, Artificial Sequence
  VH CDR1
DDYIH

SEQ ID NO: 5 - protein, 17 aa, Artificial Sequence
  VH CDR2
RIDPADGHTKYAPKFQV

SEQ ID NO: 6 - protein, 10 aa, Artificial Sequence
  VH CDR3
YGYGREVFDY

SEQ ID NO: 7 - protein, 111 aa, Artificial Sequence
  Parental Murine anti-C1s VL Variable Light
DIVLTQSPASLAVSLGQRATISCKASQSVDYDGDSYMNWYQQKTGQPPKILIYDASNLESGIPARFSGSGSGTDFTLNIHPVEEEDAAIYYCQQSNEDPWTFGGGTKLEIK

SEQ ID NO: 8 - protein, 119 aa, Artificial Sequence
  VH CDR of an anti-C1s antibody
EVQLQQSGAELVRPGASVKLSCTASGFNIKDDYIHWVKQRPEQGLEWIGRIDPADGHTKYAPKFQVKATITADTSSNTAYLQLSSLTSEDTAVYYCARYGYGREVFDYWGQGTTLTVSS

SEQ ID NO: 9 - protein, 673 aa, Artificial Sequence
  Human C1s
EPTMYGEILSPNYPQAYPSEVEKSWDIEVPEGYGIHLYFTHLDIELSENCAYDSVQIISGDTEEGRLCGQRSSNNPHSPIVEEFQVPYNKLQVIFKSDFSNEERFTGFAAYYVATDINECTDFVDVPCSHFCNNFIGGYFCSCPPEYFLHDDMKNCGVNCSGDVFTALIGEIASPNYPKPYPENSRCEYQIRLEKGFQVVVTLRREDFDVEAADSAGNCLDSLVFVAGDRQFGPYCGHGFPGPLNIETKSNALDIIFQTDLTGQKKGWKLRYHGDPMPCPKEDTPNSVWEPAKAKYVFRDVVQITCLDGFEVVEGRVGATSFYSTCQSNGKWSNSKLKCQPVDCGIPESIENGKVEDPESTLFGSVIRYTCEEPYYYMENGGGGEYHCAGNGSWVNEVLGPELPKCVPVCGVPREPFEEKQRIIGGSDADIKNFPWQVFFDNPWAGGALINEYWVLTAAHVVEGNREPTMYVGSTSVQTSRLAKSKMLTPEHVFIHPGWKLLEVPEGRTNFDNDIALVRLKDPVKMGPTVSPICLPGTSSDYNLMDGDLGLISGWGRTEKRDRAVRLKAARLPVAPLRKCKEVKVEKPTADAEAYVFTPNMICAGGEKGMDSCKGDSGGAFAVQDPNDKTKFYAAGLVSWGPQCGTYGLYTRVKNYVDWIMKTMQENSTPRED

SEQ ID NO: 10 - protein, 119 aa, Artificial Sequence
  VH1 Variant
EVQLVQSGAELKKPGASVKLSCTASGFNIKDDYIHWVKQAPGQGLEWIGRIDPADGHTKYAPKFQVKATITADTSTNTAYLQLSSLTSEDTAVYYCARYGYGREVFDYWGQGTTVTVSS

SEQ ID NO: 11 - DNA, 357 bp, Artificial Sequence
  VH variant 1
gaggttcagctggtgcagtctggggctgagcttaagaagccaggggcctcagtcaagttgtcctgcacagcttctggctttaacattaaagacgactatatacactgggtgaagcaggcccctggacagggcctggagtggattggaaggattgatcctgcggatggtcatactaaatatgccccgaagttccaagtcaaggccactataactgcagacacatccaccaacacagcctacctgcagctcagcagcctgacatctgaggacactgccgtctattactgtgctagatatggttacgggagggaggtctttgactactggggccaaggcaccactgtcacagtctcctca

SEQ ID NO: 12 - protein, 119 aa, Artificial Sequence
  VH2 variant
EVQLVQSGAEVKKPGASVKLSCTASGFNIKDDYIHWVKQAPGQGLEWIGRIDPADGHTKYAPKFQVKATITADTSTNTAYLELSSLRSEDTAVYYCARYGYGREVFDYWGQGTTVTVSS

SEQ ID NO: 13 - DNA, 357 bp, Artificial Sequence
  VH variant 2
gaggttcagctggtgcagtctggggctgaggtgaagaagccaggggcctcagtcaagttgtcctgcacagcttctggctttaacattaaagacgactatatacactgggtgaagcaggcccctggacagggcctggagtggattggaaggattgatcctgcggatggtcatactaaatatgccccgaagttccaagtcaaggccactataactgcagacacatccaccaacacagcctacctggagctcagcagcctgagatctgaggacactgccgtctattactgtgctagatatggttacgggagggaggtctttgactactggggccaaggcaccactgtcacagtctcctca

SEQ ID NO: 14 - protein, 119 aa, Artificial Sequence
  VH3 variant
QVQLVQSGAEVKKPGASVKLSCTASGFNIKDDYIHWVKQAPGQGLEWIGRIDPADGHTKYAPKFQVKVTITADTSTSTAYLELSSLRSEDTAVYYCARYGYGREVFDYWGQGTTVTVSS

SEQ ID NO: 15 - DNA, 357 bp, Artificial Sequence
  VH variant 3
caggttcagctggtgcagtctggggctgaggtgaagaagccaggggcctcagtcaagttgtcctgcacagcttctggctttaacattaaagacgactatatacactgggtgaagcaggcccctggacagggcctggagtggattggaaggattgatcctgcggatggtcatactaaatatgccccgaagttccaagtcaaagtcactataactgcagacacatccaccagcacagcctacctggagctcagcagcctgagatctgaggacactgccgtctattactgtgctagatatggttacgggagggaggtctttgactactggggccaaggcaccactgtcacagtctcctca

SEQ ID NO: 16 - protein, 119 aa, Artificial Sequence
  VH4 variant
QVQLVQSGAEVKKPGASVKVSCTASGFNIKDDYIHWVRQAPGQGLEWIGRIDPADGHTKYAPKFQVKVTITADTSTSTAYMELSSLRSEDTAVYYCARYGYGREVFDYWGQGTTVTVSS

SEQ ID NO: 17 - DNA, 357 bp, Artificial Sequence
  VH variant 4
caggttcagctggtgcagtctggggctgaggtgaagaagccaggggcctcagtcaaggtctcctgcacagcttctggctttaacattaaagacgactatatacactgggtgcgccaggcccctggacagggcctggagtggattggaaggattgatcctgcggatggtcatactaaatatgccccgaagttccaagtcaaagtcactataactgcagacacatccaccagcacagcctacatggagctcagcagcctgagatctgaggacactgccgtctattactgtgctagatatggttacgggagggaggtctttgactactggggccaaggcaccactgtcacagtctcctca

SEQ ID NO: 18 - protein, 119 aa, Artificial Sequence
  VH5 variant
QVQLVQSGAEVKKPGASVKVSCAASGFNIKDDYIHWVRQAPGQGLEWIGRIDPADGHTKYAPKFQVKVTITADTSTSTAYMELSSLRSEDTAVYYCARYGYGREVFDYWGQGTTVTVSS

SEQ ID NO: 19 - DNA, 357 bp, Artificial Sequence
  VH variant 5
caggttcagctggtgcagtctggggctgaggtgaagaagccaggggcctcagtcaaggtctcctgcgcagcttctggctttaacattaaagacgactatatacactgggtgcgccaggcccctggacagggcctggagtggattggaaggattgatcctgcggatggtcatactaaatatgccccgaagttccaagtcaaagtcactataactgcagacacatccaccagcacagcctacatggagctcagcagcctgagatctgaggacactgccgtctattactgtgctagatatggttacgggagggaggtctttgactactggggccaaggcaccactgtcacagtctcctca

SEQ ID NO: 20 - protein, 111 aa, Artificial Sequence
  Vkappa1 variant Variable Light
DIVLTQSPDSLAVSLGERATISCKASQSVDYDGDSYMNWYQQKTGQPPKILIYDASNLESGIPARFSGSGSGTDFTLTISSLEEEDFAIYYCQQSNEDPWTFGGGTKVEIK

SEQ ID NO: 21 - DNA, 333 bp, Artificial Sequence
  Vkappa variant 1
gacattgtgctgacccaatctccagactctttggctgtgtctctcggggagagggccaccatctcctgcaaggccagccaaagtgttgattatgatggtgatagttatatgaactggtaccaacaaaaaacaggacagccacccaaaatcctcatttatgatgcatccaatttggaatctggcatcccagccaggtttagtggcagtgggtctgggacagacttcaccctcaccatcagcagcctggaggaggaggattttgcaatctattactgtcagcaaagtaatgaagacccgtggacgttcggtggaggcaccaaggtggaaatcaaa

SEQ ID NO: 22 - protein, 111 aa, Artificial Sequence
  Vkappa2 variant Variable Light
DIVLTQSPDSLAVSLGERATISCKASQSVDYDGDSYMNWYQQKPGQPPKILIYDASNLESGIPARFSGSGSGTDFTLTISSLEPEDFAIYYCQQSNEDPWTFGGGTKVEIK

SEQ ID NO: 23 - DNA, 333 bp, Artificial Sequence
  Vkappa variant 2
gacattgtgctgacccaatctccagactctttggctgtgtctctcggggagagggccaccatctcctgcaaggccagccaaagtgttgattatgatggtgatagttatatgaactggtaccaacaaaaaccaggacagccacccaaaatcctcatttatgatgcatccaatttggaatctggcatcccagccaggtttagtggcagtgggtctgggacagacttcaccctcaccatcagcagcctggagcctgaggattttgcaatctattactgtcagcaaagtaatgaagacccgtggacgttcggtggaggcaccaaggtggaaatcaaa

SEQ ID NO: 24 - protein, 111 aa, Artificial Sequence
  Vkappa5 variant Variable Light
DIVLTQSPDSLAVSLGERATISCKASQSVDYDGDSYMNWYQQKPGQPPKLLIYDASNLESGIPARFSGSGSGTDFTLTISSLEPEDFAVYYCQQSNEDPWTFGGGTKVEIK

SEQ ID NO: 25 - DNA, 333 bp, Artificial Sequence
  Vkappa variant 5
gacattgtgctgacccaatctccagactctttggctgtgtctctcggggagagggccaccatctcctgcaaggccagccaaagtgttgattatgatggtgatagttatatgaactggtaccaacaaaaaccaggacagccacccaaactcctcatttatgatgcatccaatttggaatctggcatcccagccaggtttagtggcagtgggtctgggacagacttcaccctcaccatcagcagcctggagcctgaggattttgcagtctattactgtcagcaaagtaatgaagacccgtggacgttcggtggaggcaccaaggtggaaatcaaa

SEQ ID NO: 26 - protein, 119 aa, Artificial Sequence
  VH region of anti-C1s antibody
  MISC_FEATURE (1)..(1): may be Gln or Glu
  MISC_FEATURE (5)..(5): may be Val or Gln
  MISC_FEATURE (11)..(11): may be Val or Leu
  MISC_FEATURE (20)..(20): may be Leu or  Val
  MISC_FEATURE (23)..(23): may be Thr or Ala
  MISC_FEATURE (38)..(38): may be Lys or Arg
  MISC_FEATURE (68)..(68): may be Val or Ala
  MISC_FEATURE (77)..(77): may be Ser or Asn
  MISC_FEATURE (81)..(81): may be Leu or Met
  MISC_FEATURE (82)..(82): may be Glu or Gln
  MISC_FEATURE (87)..(87): may be Arg or Thr
XVQLXQSGAEXKKPGASVKXSCXASGFNIKDDYIHWVXQAPGQGLEWIGRIDPADGHTKYAPKFQVKXTITADTSTXTAYXXLSSLXSEDTAVYYCARYGYGREVFDYWGQGTTVTVSS

SEQ ID NO: 27 - protein, 111 aa, Artificial Sequence
  VL region of anti-C1s antibody
  MISC_FEATURE (44)..(44): may be Thr or Pro
  MISC_FEATURE (50)..(50): may be Ile or Leu
  MISC_FEATURE (84)..(84): may be Glu or Pro
  MISC_FEATURE (89)..(89): may be Ile or Val
DIVLTQSPDSLAVSLGERATISCKASQSVDYDGDSYMNWYQQKXGQPPKXLIYDASNLESGIPARFSGSGSGTDFTLTISSLEXEDFAXYYCQQSNEDPWTFGGGTKVEIK

SEQ ID NO: 28 - protein, 327 aa, Artificial Sequence
  Human IgG4 Constant Region (Fc) Variant 2
ASTKGPSVFPLAPCSRSTSESTAALGCLVKDYFPEPVTVSWNSGALTSGVHTFPAVLQSSGLYSLSSVVTVPSSSLGTKTYTCNVDHKPSNTKVDKRVESKYGPPCPPCPAPEFEGGPSVFLFPPKPKDTLMISRTPEVTCVVVDVSQEDPEVQFNWYVDGVEVHNAKTKPREEQFNSTYRVVSVLTVLHQDWLNGKEYKCKVSNKGLPSSIEKTISKAKGQPREPQVYTLPPSQEEMTKNQVSLTCLVKGFYPSDIAVEWESNGQPENNYKTTPPVLDSDGSFFLYSRLTVDKSRWQEGNVFSCSVLHEALHSHYTQKSLSLSLGK

SEQ ID NO: 29 - protein, 446 aa, Artificial Sequence
  VH3 Mature Heavy Chain
QVQLVQSGAEVKKPGASVKLSCTASGFNIKDDYIHWVKQAPGQGLEWIGRIDPADGHTKYAPKFQVKVTITADTSTSTAYLELSSLRSEDTAVYYCARYGYGREVFDYWGQGTTVTVSSASTKGPSVFPLAPCSRSTSESTAALGCLVKDYFPEPVTVSWNSGALTSGVHTFPAVLQSSGLYSLSSVVTVPSSSLGTKTYTCNVDHKPSNTKVDKRVESKYGPPCPPCPAPEFEGGPSVFLFPPKPKDTLMISRTPEVTCVVVDVSQEDPEVQFNWYVDGVEVHNAKTKPREEQFNSTYRVVSVLTVLHQDWLNGKEYKCKVSNKGLPSSIEKTISKAKGQPREPQVYTLPPSQEEMTKNQVSLTCLVKGFYPSDIAVEWESNGQPENNYKTTPPVLDSDGSFFLYSRLTVDKSRWQEGNVFSCSVLHEALHSHYTQKSLSLSLGK

SEQ ID NO: 30 - protein, 218 aa, Artificial Sequence
  Vkappa2 variant Mature Light Chain
DIVLTQSPDSLAVSLGERATISCKASQSVDYDGDSYMNWYQQKPGQPPKILIYDASNLESGIPARFSGSGSGTDFTLTISSLEPEDFAIYYCQQSNEDPWTFGGGTKVEIKRTVAAPSVFIFPPSDEQLKSGTASVVCLLNNFYPREAKVQWKVDNALQSGNSQESVTEQDSKDSTYSLSSTLTLSKADYEKHKVYACEVTHQGLSSPVTKSFNRGEC

SEQ ID NO: 31 - protein, 465 aa, Artificial Sequence
  synthetic amino acid sequence
MGWSLILLFLVAVATRVHSQVQLVQSGAEVKKPGASVKLSCTASGFNIKDDYIHWVKQAPGQGLEWIGRIDPADGHTKYAPKFQVKVTITADTSTSTAYLELSSLRSEDTAVYYCARYGYGREVFDYWGQGTTVTVSSASTKGPSVFPLAPCSRSTSESTAALGCLVKDYFPEPVTVSWNSGALTSGVHTFPAVLQSSGLYSLSSVVTVPSSSLGTKTYTCNVDHKPSNTKVDKRVESKYGPPCPPCPAPEFEGGPSVFLFPPKPKDTLMISRTPEVTCVVVDVSQEDPEVQFNWYVDGVEVHNAKTKPREEQFNSTYRVVSVLTVLHQDWLNGKEYKCKVSNKGLPSSIEKTISKAKGQPREPQVYTLPPSQEEMTKNQVSLTCLVKGFYPSDIAVEWESNGQPENNYKTTPPVLDSDGSFFLYSRLTVDKSRWQEGNVFSCSVLHEALHSHYTQKSLSLSLGK

SEQ ID NO: 32 - protein, 238 aa, Artificial Sequence
  synthetic amino acid sequence
MRVPAQLLGLLLLWLPGARCDIVLTQSPDSLAVSLGERATISCKASQSVDYDGDSYMNWYQQKPGQPPKILIYDASNLESGIPARFSGSGSGTDFTLTISSLEPEDFAIYYCQQSNEDPWTFGGGTKVEIKRTVAAPSVFIFPPSDEQLKSGTASVVCLLNNFYPREAKVQWKVDNALQSGNSQESVTEQDSKDSTYSLSSTLTLSKADYEKHKVYACEVTHQGLSSPVTKSFNRGEC

SEQ ID NO: 33 - protein, 11 aa, Artificial Sequence
  VL CDR1 (CDR-L1) of anti-C1s antibody
SQSVDYDGDSY

SEQ ID NO: 34 - protein, 3 aa, Artificial Sequence
  VL CDR2 (CDR-L2) of anti-C1s antibody
DAS

SEQ ID NO: 35 - protein, 6 aa, Artificial Sequence
  VL CDR3 (CDR-L3) of anti-C1s antibody
SNEDPW

SEQ ID NO: 36 - protein, 7 aa, Artificial Sequence
  VH CDR1 (CDR-H1) of anti-C1s antibody
GFNIKDD

SEQ ID NO: 37 - protein, 3 aa, Artificial Sequence
  VH CDR2 (CDR-H2) of anti-C1s antibody
ADG

SEQ ID NO: 38 - protein, 8 aa, Artificial Sequence
  VH CDR3 (CDR-H3) of anti-C1s antibody
GYGREVFD

SEQ ID NO: 39 - protein, 7 aa, Artificial Sequence
  VL CDR1 (CDR-L1) of anti-C1s antibody
DSYMNWY

SEQ ID NO: 40 - protein, 10 aa, Artificial Sequence
  VL CDR2 (CDR-L2) of anti-C1s antibody
ILIYDASNLE

SEQ ID NO: 41 - protein, 8 aa, Artificial Sequence
  VL CDR3 (CDR-L3) of anti-C1s antibody
QQSNEDPW

SEQ ID NO: 42 - protein, 6 aa, Artificial Sequence
  VH CDR1 (CDR-H1) of anti-C1s antibody
KDDYIH

SEQ ID NO: 43 - protein, 13 aa, Artificial Sequence
  VH CDR2 (CDR-H2) of anti-C1s antibody
WIGRIDPADGHTK

SEQ ID NO: 44 - protein, 11 aa, Artificial Sequence
  VH CDR3 (CDR-H3) of anti-C1s antibody
ARYGYGREVFD

SEQ ID NO: 45 - protein, 107 aa, Artificial Sequence [sequence omitted]

SEQ ID NO: 46 - protein, 446 aa, Artificial Sequence
  VH1 Mature Heavy Chain
EVQLVQSGAELKKPGASVKLSCTASGFNIKDDYIHWVKQAPGQGLEWIGRIDPADGHTKYAPKFQVKATITADTSTNTAYLQLSSLTSEDTAVYYCARYGYGREVFDYWGQGTTVTVSSASTKGPSVFPLAPCSRSTSESTAALGCLVKDYFPEPVTVSWNSGALTSGVHTFPAVLQSSGLYSLSSVVTVPSSSLGTKTYTCNVDHKPSNTKVDKRVESKYGPPCPPCPAPEFEGGPSVFLFPPKPKDTLMISRTPEVTCVVVDVSQEDPEVQFNWYVDGVEVHNAKTKPREEQFNSTYRVVSVLTVLHQDWLNGKEYKCKVSNKGLPSSIEKTISKAKGQPREPQVYTLPPSQEEMTKNQVSLTCLVKGFYPSDIAVEWESNGQPENNYKTTPPVLDSDGSFFLYSRLTVDKSRWQEGNVFSCSVLHEALHSHYTQKSLSLSLGK

SEQ ID NO: 47 - protein, 446 aa, Artificial Sequence
  VH2 Mature Heavy Chain
EVQLVQSGAEVKKPGASVKLSCTASGFNIKDDYIHWVKQAPGQGLEWIGRIDPADGHTKYAPKFQVKATITADTSTNTAYLELSSLRSEDTAVYYCARYGYGREVFDYWGQGTTVTVSSASTKGPSVFPLAPCSRSTSESTAALGCLVKDYFPEPVTVSWNSGALTSGVHTFPAVLQSSGLYSLSSVVTVPSSSLGTKTYTCNVDHKPSNTKVDKRVESKYGPPCPPCPAPEFEGGPSVFLFPPKPKDTLMISRTPEVTCVVVDVSQEDPEVQFNWYVDGVEVHNAKTKPREEQFNSTYRVVSVLTVLHQDWLNGKEYKCKVSNKGLPSSIEKTISKAKGQPREPQVYTLPPSQEEMTKNQVSLTCLVKGFYPSDIAVEWESNGQPENNYKTTPPVLDSDGSFFLYSRLTVDKSRWQEGNVFSCSVLHEALHSHYTQKSLSLSLGK

SEQ ID NO: 48 - protein, 446 aa, Artificial Sequence
  VH4 Mature Heavy Chain
QVQLVQSGAEVKKPGASVKVSCTASGFNIKDDYIHWVRQAPGQGLEWIGRIDPADGHTKYAPKFQVKVTITADTSTSTAYMELSSLRSEDTAVYYCARYGYGREVFDYWGQGTTVTVSSASTKGPSVFPLAPCSRSTSESTAALGCLVKDYFPEPVTVSWNSGALTSGVHTFPAVLQSSGLYSLSSVVTVPSSSLGTKTYTCNVDHKPSNTKVDKRVESKYGPPCPPCPAPEFEGGPSVFLFPPKPKDTLMISRTPEVTCVVVDVSQEDPEVQFNWYVDGVEVHNAKTKPREEQFNSTYRVVSVLTVLHQDWLNGKEYKCKVSNKGLPSSIEKTISKAKGQPREPQVYTLPPSQEEMTKNQVSLTCLVKGFYPSDIAVEWESNGQPENNYKTTPPVLDSDGSFFLYSRLTVDKSRWQEGNVFSCSVLHEALHSHYTQKSLSLSLGK

SEQ ID NO: 49 - protein, 446 aa, Artificial Sequence
  VH5 Mature Heavy Chain
QVQLVQSGAEVKKPGASVKVSCAASGFNIKDDYIHWVRQAPGQGLEWIGRIDPADGHTKYAPKFQVKVTITADTSTSTAYMELSSLRSEDTAVYYCARYGYGREVFDYWGQGTTVTVSSASTKGPSVFPLAPCSRSTSESTAALGCLVKDYFPEPVTVSWNSGALTSGVHTFPAVLQSSGLYSLSSVVTVPSSSLGTKTYTCNVDHKPSNTKVDKRVESKYGPPCPPCPAPEFEGGPSVFLFPPKPKDTLMISRTPEVTCVVVDVSQEDPEVQFNWYVDGVEVHNAKTKPREEQFNSTYRVVSVLTVLHQDWLNGKEYKCKVSNKGLPSSIEKTISKAKGQPREPQVYTLPPSQEEMTKNQVSLTCLVKGFYPSDIAVEWESNGQPENNYKTTPPVLDSDGSFFLYSRLTVDKSRWQEGNVFSCSVLHEALHSHYTQKSLSLSLGK

SEQ ID NO: 50 - protein, 218 aa, Artificial Sequence
  Vkappa1 variant Mature Light Chain
DIVLTQSPDSLAVSLGERATISCKASQSVDYDGDSYMNWYQQKTGQPPKILIYDASNLESGIPARFSGSGSGTDFTLTISSLEEEDFAIYYCQQSNEDPWTFGGGTKVEIKRTVAAPSVFIFPPSDEQLKSGTASVVCLLNNFYPREAKVQWKVDNALQSGNSQESVTEQDSKDSTYSLSSTLTLSKADYEKHKVYACEVTHQGLSSPVTKSFNRGEC

SEQ ID NO: 51 - protein, 218 aa, Artificial Sequence
  Vkappa5 variant Mature Light Chain
DIVLTQSPDSLAVSLGERATISCKASQSVDYDGDSYMNWYQQKPGQPPKLLIYDASNLESGIPARFSGSGSGTDFTLTISSLEPEDFAVYYCQQSNEDPWTFGGGTKVEIKRTVAAPSVFIFPPSDEQLKSGTASVVCLLNNFYPREAKVQWKVDNALQSGNSQESVTEQDSKDSTYSLSSTLTLSKADYEKHKVYACEVTHQGLSSPVTKSFNRGEC

SEQ ID NO: 52 - protein, 327 aa, Artificial Sequence
  Human IgG4 Constant Region (Fc)
ASTKGPSVFPLAPCSRSTSESTAALGCLVKDYFPEPVTVSWNSGALTSGVHTFPAVLQSSGLYSLSSVVTVPSSSLGTKTYTCNVDHKPSNTKVDKRVESKYGPPCPSCPAPEFLGGPSVFLFPPKPKDTLMISRTPEVTCVVVDVSQEDPEVQFNWYVDGVEVHNAKTKPREEQFNSTYRVVSVLTVLHQDWLNGKEYKCKVSNKGLPSSIEKTISKAKGQPREPQVYTLPPSQEEMTKNQVSLTCLVKGFYPSDIAVEWESNGQPENNYKTTPPVLDSDGSFFLYSRLTVDKSRWQEGNVFSCSVMHEALHNHYTQKSLSLSLGK

SEQ ID NO: 53 - protein, 327 aa, Artificial Sequence
  Human IgG4 Constant Region (Fc) Variant 1
ASTKGPSVFPLAPCSRSTSESTAALGCLVKDYFPEPVTVSWNSGALTSGVHTFPAVLQSSGLYSLSSVVTVPSSSLGTKTYTCNVDHKPSNTKVDKRVESKYGPPCPPCPAPEFEGGPSVFLFPPKPKDTLMISRTPEVTCVVVDVSQEDPEVQFNWYVDGVEVHNAKTKPREEQFNSTYRVVSVLTVLHQDWLNGKEYKCKVSNKGLPSSIEKTISKAKGQPREPQVYTLPPSQEEMTKNQVSLTCLVKGFYPSDIAVEWESNGQPENNYKTTPPVLDSDGSFFLYSRLTVDKSRWQEGNVFSCSVMHEALHNHYTQKSLSLSLGK

SEQ ID NO: 54 - protein, 218 aa, Artificial Sequence
  Parental Murine anti-C1s VL Mature Light Chain
DIVLTQSPASLAVSLGQRATISCKASQSVDYDGDSYMNWYQQKTGQPPKILIYDASNLESGIPARFSGSGSGTDFTLNIHPVEEEDAAIYYCQQSNEDPWTFGGGTKLEIKRTVAAPSVFIFPPSDEQLKSGTASVVCLLNNFYPREAKVQWKVDNALQSGNSQESVTEQDSKDSTYSLSSTLTLSKADYEKHKVYACEVTHQGLSSPVTKSFNRGEC